European Patent Application EP 4 365 303 A1, published May 8, 2024. Title: Purification of linear DNA products. Applicant: 4basebio, S.L.U. Application EP. The sequence listing filed with the application follows.

SEQUENCE LISTING (10 sequences)

SEQ ID NO: 1 - DNA, 20 bp, synthetic construct
  source 1..20: mol_type = other DNA
  modified_base 6: mod_base = OTHER; note = biotinylated
  modified_base 11: mod_base = OTHER; note = biotinylated
  modified_base 16: mod_base = OTHER; note = biotinylated
agggctaacatttgttggcc

SEQ ID NO: 2 - DNA, 20 bp, synthetic construct
  source 1..20: mol_type = other DNA
  modified_base 11: mod_base = OTHER; note = biotinylated
  modified_base 16: mod_base = OTHER; note = biotinylated
agggctaacatttgttggcc

SEQ ID NO: 3 - DNA, 20 bp, synthetic construct
  source 1..20: mol_type = other DNA
  modified_base 16: mod_base = OTHER; note = biotinylated
agggctaacatttgttggcc

SEQ ID NO: 4 - DNA, 16 bp, synthetic construct
  source 1..16: mol_type = other DNA
  modified_base 1..5: mod_base = OTHER; note = phoshphorothioated
ggccaacaaatgttag

SEQ ID NO: 5 - DNA, 14 bp, synthetic construct
  source 1..14: mol_type = other DNA
  modified_base 1: mod_base = OTHER; note = biotinylated
tttttttttttttt

SEQ ID NO: 6 - DNA, 14 bp, synthetic construct
  source 1..14: mol_type = other DNA
  modified_base 1: mod_base = OTHER; note = biotinylated
  modified_base 6: mod_base = OTHER; note = biotinylated
tttttttttttttt

SEQ ID NO: 7 - DNA, 14 bp, synthetic construct
  source 1..14: mol_type = other DNA
  modified_base 1: mod_base = OTHER; note = biotinylated
  modified_base 6: mod_base = OTHER; note = biotinylated
  modified_base 11: mod_base = OTHER; note = biotinylated
tttttttttttttt

SEQ ID NO: 8 - DNA, 18 bp, synthetic construct
  source 1..18: mol_type = other DNA
  modified_base 14..18: mod_base = OTHER; note = phosphorothioated
aaaaaaaaaaaaaaaaaa

SEQ ID NO: 9 - DNA, 41 bp, synthetic construct
  source 1..41: mol_type = other DNA
  modified_base 16: mod_base = OTHER; note = biotinylated
  modified_base 21: mod_base = OTHER; note = biotinylated
  modified_base 23: mod_base = OTHER; note = biotinylated
  modified_base 25: mod_base = OTHER; note = biotinylated
  modified_base 31: mod_base = OTHER; note = biotinylated
agggagtctccttgatggcctctctggccatcaaggagact

SEQ ID NO: 10 - DNA, 41 bp, synthetic construct
  source 1..41: mol_type = other DNA
  modified_base 23: mod_base = OTHER; note = biotinylated
agggagtctccttgttggccactcaggccaacaaggagact